European Patent Application EP 4 624 499 A1, published October 1, 2025. Title: T-CELL ANTIGEN RECEPTOR, PREPARATION METHOD THEREFOR, AND USE THEREOF. Applicant: 北京永泰瑞科生物科技有限公司. Application EP 23905913.2, filed June 23, 2025. The sequence listing filed with the application follows.

SEQUENCE LISTING (111 sequences)

SEQ ID NO: 1 - protein, 6 aa, synthetic construct
SSNFYA

SEQ ID NO: 2 - protein, 7 aa, synthetic construct
MTLNGDE

SEQ ID NO: 3 - protein, 10 aa, synthetic construct
CARNTGKLIF

SEQ ID NO: 4 - protein, 5 aa, synthetic construct
SQVTM

SEQ ID NO: 5 - protein, 7 aa, synthetic construct
ANQGSEA

SEQ ID NO: 6 - protein, 14 aa, synthetic construct
CSANPTGGGTEAFF

SEQ ID NO: 7 - protein, 109 aa, synthetic construct
ILNVEQSPQSLHVQEGDSTNFTCSFPSSNFYALHWYRWETAKSPEALFVMTLNGDEKKKGRISATLNTKEGYSYLYIKGSQPEDSATYLCARNTGKLIFGQGTTLQVKP

SEQ ID NO: 8 - protein, 114 aa, synthetic construct
AVISQKPSRDICQRGTSLTIQCQVDSQVTMMFWYRQQPGQSLTLIATANQGSEATYESGFVIDKFPISRPNLTFSTLTVSNMSPEDSSIYLCSANPTGGGTEAFFGQGTRLTVV

SEQ ID NO: 9 - protein, 272 aa, synthetic construct
MEKNPLAAPLLILWFHLDCVSSILNVEQSPQSLHVQEGDSTNFTCSFPSSNFYALHWYRWETAKSPEALFVMTLNGDEKKKGRISATLNTKEGYSYLYIKGSQPEDSATYLCARNTGKLIFGQGTTLQVKPDIQNPDPAVYQLRDSKSSDKSVCLFTDFDSQTNVSQSKDSDVYITDKTVLDMRSMDFKSNSAVAWSNKSDFACANAFNNSIIPEDTFFPSPESSCDVKLVEKSFETDTNLNFQNLSVIGFRILLLKVAGFNLLMTLRLWSS

SEQ ID NO: 10 - protein, 307 aa, synthetic construct
MLSLLLLLLGLGSVFSAVISQKPSRDICQRGTSLTIQCQVDSQVTMMFWYRQQPGQSLTLIATANQGSEATYESGFVIDKFPISRPNLTFSTLTVSNMSPEDSSIYLCSANPTGGGTEAFFGQGTRLTVVEDLNKVFPPEVAVFEPSEAEISHTQKATLVCLATGFFPDHVELSWWVNGKEVHSGVSTDPQPLKEQPALNDSRYCLSSRLRVSATFWQNPRNHFRCQVQFYGLSENDEWTQDRAKPVTQIVSAEAWGRADCGFTSVSYQQGVLSATILYEILLGKATLYAVLVSALVLMAMVKRKDF

SEQ ID NO: 11 - protein, 27 aa, synthetic construct
RAKRSGSGATNFSLLKQAGDVEENPGP

SEQ ID NO: 12 - protein, 606 aa, synthetic construct
MEKNPLAAPLLILWFHLDCVSSILNVEQSPQSLHVQEGDSTNFTCSFPSSNFYALHWYRWETAKSPEALFVMTLNGDEKKKGRISATLNTKEGYSYLYIKGSQPEDSATYLCARNTGKLIFGQGTTLQVKPDIQNPDPAVYQLRDSKSSDKSVCLFTDFDSQTNVSQSKDSDVYITDKTVLDMRSMDFKSNSAVAWSNKSDFACANAFNNSIIPEDTFFPSPESSCDVKLVEKSFETDTNLNFQNLSVIGFRILLLKVAGFNLLMTLRLWSSRAKRSGSGATNFSLLKQAGDVEENPGPMLSLLLLLLGLGSVFSAVISQKPSRDICQRGTSLTIQCQVDSQVTMMFWYRQQPGQSLTLIATANQGSEATYESGFVIDKFPISRPNLTFSTLTVSNMSPEDSSIYLCSANPTGGGTEAFFGQGTRLTVVEDLNKVFPPEVAVFEPSEAEISHTQKATLVCLATGFFPDHVELSWWVNGKEVHSGVSTDPQPLKEQPALNDSRYCLSSRLRVSATFWQNPRNHFRCQVQFYGLSENDEWTQDRAKPVTQIVSAEAWGRADCGFTSVSYQQGVLSATILYEILLGKATLYAVLVSALVLMAMVKRKDF

SEQ ID NO: 13 - protein, 9 aa, synthetic construct
QYDPVAALF

SEQ ID NO: 14 - protein, 5 aa, synthetic construct
SGHVS

SEQ ID NO: 15 - protein, 6 aa, synthetic construct
FQNEAQ

SEQ ID NO: 16 - protein, 14 aa, synthetic construct
CASSLLTRTETQYF

SEQ ID NO: 17 - protein, 109 aa, synthetic construct; identical to SEQ ID NO: 7

SEQ ID NO: 18 - protein, 109 aa, synthetic construct
QSPRYKVAKRGQDVALRCDPISGHVSLFWYQQALGQGPEFLTYFQNEAQLDKSGLPSDRFFAERPEGSVSTLKIQRTQQEDSAVYLCASSLLTRTETQYFGPGTRLLVL

SEQ ID NO: 19 - protein, 272 aa, synthetic construct; identical to SEQ ID NO: 9

SEQ ID NO: 20 - protein, 310 aa, synthetic construct
MGTRLLCWVVLGFLGTDHTGAGVSQSPRYKVAKRGQDVALRCDPISGHVSLFWYQQALGQGPEFLTYFQNEAQLDKSGLPSDRFFAERPEGSVSTLKIQRTQQEDSAVYLCASSLLTRTETQYFGPGTRLLVLEDLKNVFPPEVAVFEPSEAEISHTQKATLVCLATGFYPDHVELSWWVNGKEVHSGVSTDPQPLKEQPALNDSRYCLSSRLRVSATFWQNPRNHFRCQVQFYGLSENDEWTQDRAKPVTQIVSAEAWGRADCGFTSESYQQGVLSATILYEILLGKATLYAVLVSALVLMAMVKRKDF

SEQ ID NO: 21 - protein, 609 aa, synthetic construct
MEKNPLAAPLLILWFHLDCVSSILNVEQSPQSLHVQEGDSTNFTCSFPSSNFYALHWYRWETAKSPEALFVMTLNGDEKKKGRISATLNTKEGYSYLYIKGSQPEDSATYLCARNTGKLIFGQGTTLQVKPDIQNPDPAVYQLRDSKSSDKSVCLFTDFDSQTNVSQSKDSDVYITDKTVLDMRSMDFKSNSAVAWSNKSDFACANAFNNSIIPEDTFFPSPESSCDVKLVEKSFETDTNLNFQNLSVIGFRILLLKVAGFNLLMTLRLWSSRAKRSGSGATNFSLLKQAGDVEENPGPMGTRLLCWVVLGFLGTDHTGAGVSQSPRYKVAKRGQDVALRCDPISGHVSLFWYQQALGQGPEFLTYFQNEAQLDKSGLPSDRFFAERPEGSVSTLKIQRTQQEDSAVYLCASSLLTRTETQYFGPGTRLLVLEDLKNVFPPEVAVFEPSEAEISHTQKATLVCLATGFYPDHVELSWWVNGKEVHSGVSTDPQPLKEQPALNDSRYCLSSRLRVSATFWQNPRNHFRCQVQFYGLSENDEWTQDRAKPVTQIVSAEAWGRADCGFTSESYQQGVLSATILYEILLGKATLYAVLVSALVLMAMVKRKDF

SEQ ID NO: 22 - protein, 10 aa, synthetic construct
CAPSASKIIF

SEQ ID NO: 23 - protein, 5 aa, synthetic construct
LNHDA

SEQ ID NO: 24 - protein, 6 aa, synthetic construct
SQIVND

SEQ ID NO: 25 - protein, 18 aa, synthetic construct
CASSTTGLAGGPGNEQFF

SEQ ID NO: 26 - protein, 113 aa, synthetic construct
CVSSILNVEQSPQSLHVQEGDSTNFTCSFPSSNFYALHWYRWETAKSPEALFVMTLNGDEKKKGRISATLNTKEGYSYLYIKGSQPEDSATYLCAPSASKIIFGSGTRLSIRP

SEQ ID NO: 27 - protein, 120 aa, synthetic construct
NTVDGGITQSPKYLFRKEGQNVTLSCEQNLNHDAMYWYRQDPGQGLRLIYYSQIVNDFQKGDIAEGYSVSREKKESFPLTVTSAQKNPTAFYLCASSTTGLAGGPGNEQFFGPGTRLTVL

SEQ ID NO: 28 - protein, 272 aa, synthetic construct
MEKNPLAAPLLILWFHLDCVSSILNVEQSPQSLHVQEGDSTNFTCSFPSSNFYALHWYRWETAKSPEALFVMTLNGDEKKKGRISATLNTKEGYSYLYIKGSQPEDSATYLCAPSASKIIFGSGTRLSIRPNIQNPDPAVYQLRDSKSSDKSVCLFTDFDSQTNVSQSKDSDVYITDKTVLDMRSMDFKSNSAVAWSNKSDFACANAFNNSIIPEDTFFPSPESSCDVKLVEKSFETDTNLNFQNLSVIGFRILLLKVAGFNLLMTLRLWSS

SEQ ID NO: 29 - protein, 313 aa, synthetic construct
MSNQVLCCVVLCLLGANTVDGGITQSPKYLFRKEGQNVTLSCEQNLNHDAMYWYRQDPGQGLRLIYYSQIVNDFQKGDIAEGYSVSREKKESFPLTVTSAQKNPTAFYLCASSTTGLAGGPGNEQFFGPGTRLTVLEDLKNVFPPEVAVFEPSEAEISHTQKATLVCLATGFFPDHVELSWWVNGKEVHSGVSTDPQPLKEQPALNDSRYCLSSRLRVSATFWQNPRNHFRCQVQFYGLSENDEWTQDRAKPVTQIVSAEAWGRADCGFTSESYQQGVLSATILYEILLGKATLYAVLVSALVLMAMVKRKDF

SEQ ID NO: 30 - protein, 612 aa, synthetic construct
MEKNPLAAPLLILWFHLDCVSSILNVEQSPQSLHVQEGDSTNFTCSFPSSNFYALHWYRWETAKSPEALFVMTLNGDEKKKGRISATLNTKEGYSYLYIKGSQPEDSATYLCAPSASKIIFGSGTRLSIRPNIQNPDPAVYQLRDSKSSDKSVCLFTDFDSQTNVSQSKDSDVYITDKTVLDMRSMDFKSNSAVAWSNKSDFACANAFNNSIIPEDTFFPSPESSCDVKLVEKSFETDTNLNFQNLSVIGFRILLLKVAGFNLLMTLRLWSSRAKRSGSGATNFSLLKQAGDVEENPGPMSNQVLCCVVLCLLGANTVDGGITQSPKYLFRKEGQNVTLSCEQNLNHDAMYWYRQDPGQGLRLIYYSQIVNDFQKGDIAEGYSVSREKKESFPLTVTSAQKNPTAFYLCASSTTGLAGGPGNEQFFGPGTRLTVLEDLKNVFPPEVAVFEPSEAEISHTQKATLVCLATGFFPDHVELSWWVNGKEVHSGVSTDPQPLKEQPALNDSRYCLSSRLRVSATFWQNPRNHFRCQVQFYGLSENDEWTQDRAKPVTQIVSAEAWGRADCGFTSESYQQGVLSATILYEILLGKATLYAVLVSALVLMAMVKRKDF

SEQ ID NO: 31 - protein, 10 aa, synthetic construct
CAPQFNKFYF

SEQ ID NO: 32 - protein, 113 aa, synthetic construct
CVSSILNVEQSPQSLHVQEGDSTNFTCSFPSSNFYALHWYRWETAKSPEALFVMTLNGDEKKKGRISATLNTKEGYSYLYIKGSQPEDSATYLCAPQFNKFYFGSGTKLNVKP

SEQ ID NO: 33 - protein, 117 aa, synthetic construct
DHTGAGVSQSPRYKVAKRGQDVALRCDPISGHVSLFWYQQALGQGPEFLTYFQNEAQLDKSGLPSDRFFAERPEGSVSTLKIQRTQQEDSAVYLCASSLLTRTETQYFGPGTRLLVL

SEQ ID NO: 34 - protein, 272 aa, synthetic construct
MEKNPLAAPLLILWFHLDCVSSILNVEQSPQSLHVQEGDSTNFTCSFPSSNFYALHWYRWETAKSPEALFVMTLNGDEKKKGRISATLNTKEGYSYLYIKGSQPEDSATYLCAPQFNKFYFGSGTKLNVKPNIQNPDPAVYQLRDSKSSDKSVCLFTDFDSQTNVSQSKDSDVYITDKTVLDMRSMDFKSNSAVAWSNKSDFACANAFNNSIIPEDTFFPSPESSCDVKLVEKSFETDTNLNFQNLSVIGFRILLLKVAGFNLLMTLRLWSS

SEQ ID NO: 35 - protein, 310 aa, synthetic construct; identical to SEQ ID NO: 20

SEQ ID NO: 36 - protein, 609 aa, synthetic construct
MEKNPLAAPLLILWFHLDCVSSILNVEQSPQSLHVQEGDSTNFTCSFPSSNFYALHWYRWETAKSPEALFVMTLNGDEKKKGRISATLNTKEGYSYLYIKGSQPEDSATYLCAPQFNKFYFGSGTKLNVKPNIQNPDPAVYQLRDSKSSDKSVCLFTDFDSQTNVSQSKDSDVYITDKTVLDMRSMDFKSNSAVAWSNKSDFACANAFNNSIIPEDTFFPSPESSCDVKLVEKSFETDTNLNFQNLSVIGFRILLLKVAGFNLLMTLRLWSSRAKRSGSGATNFSLLKQAGDVEENPGPMGTRLLCWVVLGFLGTDHTGAGVSQSPRYKVAKRGQDVALRCDPISGHVSLFWYQQALGQGPEFLTYFQNEAQLDKSGLPSDRFFAERPEGSVSTLKIQRTQQEDSAVYLCASSLLTRTETQYFGPGTRLLVLEDLKNVFPPEVAVFEPSEAEISHTQKATLVCLATGFYPDHVELSWWVNGKEVHSGVSTDPQPLKEQPALNDSRYCLSSRLRVSATFWQNPRNHFRCQVQFYGLSENDEWTQDRAKPVTQIVSAEAWGRADCGFTSESYQQGVLSATILYEILLGKATLYAVLVSALVLMAMVKRKDF

SEQ ID NO: 37 - protein, 11 aa, synthetic construct
CASINFNKFYF

SEQ ID NO: 38 - protein, 5 aa, synthetic construct
MDHEN

SEQ ID NO: 39 - protein, 6 aa, synthetic construct
SYDVKM

SEQ ID NO: 40 - protein, 15 aa, synthetic construct
CASSPLNGGATEAFF

SEQ ID NO: 41 - protein, 110 aa, synthetic construct
ILNVEQSPQSLHVQEGDSTNFTCSFPSSNFYALHWYRWETAKSPEALFVMTLNGDEKKKGRISATLNTKEGYSYLYIKGSQPEDSATYLCASINFNKFYFGSGTKLNVKP

SEQ ID NO: 42 - protein, 107 aa, synthetic construct
SRYLVKRTGEKVFLECVQDMDHENMFWYRQDPGLGLRLIYFSYDVKMKEKGDIPEGYSVSREKKERFSLILESASTNQTSMYLCASSPLNGGATEAFFGQGTRLTVV

SEQ ID NO: 43 - protein, 273 aa, synthetic construct
MEKNPLAAPLLILWFHLDCVSSILNVEQSPQSLHVQEGDSTNFTCSFPSSNFYALHWYRWETAKSPEALFVMTLNGDEKKKGRISATLNTKEGYSYLYIKGSQPEDSATYLCASINFNKFYFGSGTKLNVKPNIQNPDPAVYQLRDSKSSDKSVCLFTDFDSQTNVSQSKDSDVYITDKTVLDMRSMDFKSNSAVAWSNKSDFACANAFNNSIIPEDTFFPSPESSCDVKLVEKSFETDTNLNFQNLSVIGFRILLLKVAGFNLLMTLRLWSS

SEQ ID NO: 44 - protein, 310 aa, synthetic construct
MGIRLLCRVAFCFLAVGLVDVKVTQSSRYLVKRTGEKVFLECVQDMDHENMFWYRQDPGLGLRLIYFSYDVKMKEKGDIPEGYSVSREKKERFSLILESASTNQTSMYLCASSPLNGGATEAFFGQGTRLTVVEDLNKVFPPEVAVFEPSEAEISHTQKATLVCLATGFFPDHVELSWWVNGKEVHSGVSTDPQPLKEQPALNDSRYCLSSRLRVSATFWQNPRNHFRCQVQFYGLSENDEWTQDRAKPVTQIVSAEAWGRADCGFTSVSYQQGVLSATILYEILLGKATLYAVLVSALVLMAMVKRKDF

SEQ ID NO: 45 - protein, 610 aa, synthetic construct
MEKNPLAAPLLILWFHLDCVSSILNVEQSPQSLHVQEGDSTNFTCSFPSSNFYALHWYRWETAKSPEALFVMTLNGDEKKKGRISATLNTKEGYSYLYIKGSQPEDSATYLCASINFNKFYFGSGTKLNVKPNIQNPDPAVYQLRDSKSSDKSVCLFTDFDSQTNVSQSKDSDVYITDKTVLDMRSMDFKSNSAVAWSNKSDFACANAFNNSIIPEDTFFPSPESSCDVKLVEKSFETDTNLNFQNLSVIGFRILLLKVAGFNLLMTLRLWSSRAKRSGSGATNFSLLKQAGDVEENPGPMGIRLLCRVAFCFLAVGLVDVKVTQSSRYLVKRTGEKVFLECVQDMDHENMFWYRQDPGLGLRLIYFSYDVKMKEKGDIPEGYSVSREKKERFSLILESASTNQTSMYLCASSPLNGGATEAFFGQGTRLTVVEDLNKVFPPEVAVFEPSEAEISHTQKATLVCLATGFFPDHVELSWWVNGKEVHSGVSTDPQPLKEQPALNDSRYCLSSRLRVSATFWQNPRNHFRCQVQFYGLSENDEWTQDRAKPVTQIVSAEAWGRADCGFTSVSYQQGVLSATILYEILLGKATLYAVLVSALVLMAMVKRKDF

SEQ ID NO: 46 - protein, 9 aa, synthetic construct
NLVPMVATV

SEQ ID NO: 47 - protein, 6 aa, synthetic construct
DSSSTY

SEQ ID NO: 48 - protein, 7 aa, synthetic construct
IFSNMDM

SEQ ID NO: 49 - protein, 13 aa, synthetic construct
CAEFTGTASKLTF

SEQ ID NO: 50 - protein, 6 aa, synthetic construct
GTSNPN

SEQ ID NO: 51 - protein, 5 aa, synthetic construct
SVGIG

SEQ ID NO: 52 - protein, 15 aa, synthetic construct
CAWSDRAAFTDTQYF

SEQ ID NO: 53 - protein, 115 aa, synthetic construct
CMSRGEDVEQSLFLSVREGDSSVINCTYTDSSSTYLYWYKQEPGAGLQLLTYIFSNMDMKQDQRLTVLLNKKDKHLSLRIADTQTGDSAIYFCAEFTGTASKLTFGTGTRLQVTL

SEQ ID NO: 54 - protein, 117 aa, synthetic construct
GVRSQTIHQWPATLVQPVGSPLSLECTVEGTSNPNLYWYRQAAGRGLQLLFYSVGIGQISSEVPQNLSASRPQDRQFILSSKKLLLSDSGFYLCAWSDRAAFTDTQYFGPGTRLTVL

SEQ ID NO: 55 - protein, 273 aa, synthetic construct
MKTFAGFSFLFLWLQLDCMSRGEDVEQSLFLSVREGDSSVINCTYTDSSSTYLYWYKQEPGAGLQLLTYIFSNMDMKQDQRLTVLLNKKDKHLSLRIADTQTGDSAIYFCAEFTGTASKLTFGTGTRLQVTLDIQNPDPAVYQLRDSKSSDKSVCLFTDFDSQTNVSQSKDSDVYITDKTVLDMRSMDFKSNSAVAWSNKSDFACANAFNNSIIPEDTFFPSPESSCDVKLVEKSFETDTNLNFQNLSVIGFRILLLKVAGFNLLMTLRLWSS

SEQ ID NO: 56 - protein, 308 aa, synthetic construct
MLCSLLALLLGTFFGVRSQTIHQWPATLVQPVGSPLSLECTVEGTSNPNLYWYRQAAGRGLQLLFYSVGIGQISSEVPQNLSASRPQDRQFILSSKKLLLSDSGFYLCAWSDRAAFTDTQYFGPGTRLTVLEDLKNVFPPEVAVFEPSEAEISHTQKATLVCLATGFYPDHVELSWWVNGKEVHSGVSTDPQPLKEQPALNDSRYCLSSRLRVSATFWQNPRNHFRCQVQFYGLSENDEWTQDRAKPVTQIVSAEAWGRADCGFTSESYQQGVLSATILYEILLGKATLYAVLVSALVLMAMVKRKDF

SEQ ID NO: 57 - protein, 608 aa, synthetic construct
MKTFAGFSFLFLWLQLDCMSRGEDVEQSLFLSVREGDSSVINCTYTDSSSTYLYWYKQEPGAGLQLLTYIFSNMDMKQDQRLTVLLNKKDKHLSLRIADTQTGDSAIYFCAEFTGTASKLTFGTGTRLQVTLDIQNPDPAVYQLRDSKSSDKSVCLFTDFDSQTNVSQSKDSDVYITDKTVLDMRSMDFKSNSAVAWSNKSDFACANAFNNSIIPEDTFFPSPESSCDVKLVEKSFETDTNLNFQNLSVIGFRILLLKVAGFNLLMTLRLWSSRAKRSGSGATNFSLLKQAGDVEENPGPMLCSLLALLLGTFFGVRSQTIHQWPATLVQPVGSPLSLECTVEGTSNPNLYWYRQAAGRGLQLLFYSVGIGQISSEVPQNLSASRPQDRQFILSSKKLLLSDSGFYLCAWSDRAAFTDTQYFGPGTRLTVLEDLKNVFPPEVAVFEPSEAEISHTQKATLVCLATGFYPDHVELSWWVNGKEVHSGVSTDPQPLKEQPALNDSRYCLSSRLRVSATFWQNPRNHFRCQVQFYGLSENDEWTQDRAKPVTQIVSAEAWGRADCGFTSESYQQGVLSATILYEILLGKATLYAVLVSALVLMAMVKRKDF

SEQ ID NO: 58 - protein, 6 aa, synthetic construct
TSGFNG

SEQ ID NO: 59 - protein, 6 aa, synthetic construct
NVLDGL

SEQ ID NO: 60 - protein, 12 aa, synthetic construct
CAVTYNNARLMF

SEQ ID NO: 61 - protein, 5 aa, synthetic construct
MNHEY

SEQ ID NO: 62 - protein, 6 aa, synthetic construct
SMNVEV

SEQ ID NO: 63 - protein, 15 aa, synthetic construct
CASSSVAGGRIEQFF

SEQ ID NO: 64 - protein, 112 aa, synthetic construct
GTTGQNIDQPTEMTATEGAIVQINCTYQTSGFNGLFWYQQHAGEAPTFLSYNVLDGLEEKGRFSSFLSRSKGYSYLLLKELQMKDSASYLCAVTYNNARLMFGDGTQLVVKP

SEQ ID NO: 65 - protein, 117 aa, synthetic construct
GPLEAQVTQNPRYLITVTGKKLTVTCSQNMNHEYMSWYRQDPGLGLRQIYYSMNVEVTDKGDVPEGYKVSRKEKRNFPLILESPSPNQTSLYFCASSSVAGGRIEQFFGPGTRLTVL

SEQ ID NO: 66 - protein, 267 aa, synthetic construct
MWGVFLLYVSMKMGGTTGQNIDQPTEMTATEGAIVQINCTYQTSGFNGLFWYQQHAGEAPTFLSYNVLDGLEEKGRFSSFLSRSKGYSYLLLKELQMKDSASYLCAVTYNNARLMFGDGTQLVVKPNIQNPDPAVYQLRDSKSSDKSVCLFTDFDSQTNVSQSKDSDVYITDKTVLDMRSMDFKSNSAVAWSNKSDFACANAFNNSIIPEDTFFPSPESSCDVKLVEKSFETDTNLNFQNLSVIGFRILLLKVAGFNLLMTLRLWSS

SEQ ID NO: 67 - protein, 310 aa, synthetic construct
MGPQLLGYVVLCLLGAGPLEAQVTQNPRYLITVTGKKLTVTCSQNMNHEYMSWYRQDPGLGLRQIYYSMNVEVTDKGDVPEGYKVSRKEKRNFPLILESPSPNQTSLYFCASSSVAGGRIEQFFGPGTRLTVLEDLKNVFPPEVAVFEPSEAEISHTQKATLVCLATGFYPDHVELSWWVNGKEVHSGVSTDPQPLKEQPALNDSRYCLSSRLRVSATFWQNPRNHFRCQVQFYGLSENDEWTQDRAKPVTQIVSAEAWGRADCGFTSESYQQGVLSATILYEILLGKATLYAVLVSALVLMAMVKRKDF

SEQ ID NO: 68 - protein, 604 aa, synthetic construct
MWGVFLLYVSMKMGGTTGQNIDQPTEMTATEGAIVQINCTYQTSGFNGLFWYQQHAGEAPTFLSYNVLDGLEEKGRFSSFLSRSKGYSYLLLKELQMKDSASYLCAVTYNNARLMFGDGTQLVVKPNIQNPDPAVYQLRDSKSSDKSVCLFTDFDSQTNVSQSKDSDVYITDKTVLDMRSMDFKSNSAVAWSNKSDFACANAFNNSIIPEDTFFPSPESSCDVKLVEKSFETDTNLNFQNLSVIGFRILLLKVAGFNLLMTLRLWSSRAKRSGSGATNFSLLKQAGDVEENPGPMGPQLLGYVVLCLLGAGPLEAQVTQNPRYLITVTGKKLTVTCSQNMNHEYMSWYRQDPGLGLRQIYYSMNVEVTDKGDVPEGYKVSRKEKRNFPLILESPSPNQTSLYFCASSSVAGGRIEQFFGPGTRLTVLEDLKNVFPPEVAVFEPSEAEISHTQKATLVCLATGFYPDHVELSWWVNGKEVHSGVSTDPQPLKEQPALNDSRYCLSSRLRVSATFWQNPRNHFRCQVQFYGLSENDEWTQDRAKPVTQIVSAEAWGRADCGFTSESYQQGVLSATILYEILLGKATLYAVLVSALVLMAMVKRKDF

SEQ ID NO: 69 - protein, 11 aa, synthetic construct
CARNYGQNFVF

SEQ ID NO: 70 - protein, 6 aa, synthetic construct
DFQATT

SEQ ID NO: 71 - protein, 7 aa, synthetic construct
SNEGSKA

SEQ ID NO: 72 - protein, 16 aa, synthetic construct
CSARDIKAQQWNIQYF

SEQ ID NO: 73 - protein, 114 aa, synthetic construct
CVSSILNVEQSPQSLHVQEGDSTNFTCSFPSSNFYALHWYRWETAKSPEALFVMTLNGDEKKKGRISATLNTKEGYSYLYIKGSQPEDSATYLCARNYGQNFVFGPGTRLSVLP

SEQ ID NO: 74 - protein, 122 aa, synthetic construct
GSGLGAVVSQHPSWVICKSGTSVKIECRSLDFQATTMFWYRQFPKQSLMLMATSNEGSKATYEQGVEKDKFLINHASLTLSTLTVTSAHPEDSSFYICSARDIKAQQWNIQYFGAGTRLSVL

SEQ ID NO: 75 - protein, 273 aa, synthetic construct
MEKNPLAAPLLILWFHLDCVSSILNVEQSPQSLHVQEGDSTNFTCSFPSSNFYALHWYRWETAKSPEALFVMTLNGDEKKKGRISATLNTKEGYSYLYIKGSQPEDSATYLCARNYGQNFVFGPGTRLSVLPYIQNPDPAVYQLRDSKSSDKSVCLFTDFDSQTNVSQSKDSDVYITDKTVLDMRSMDFKSNSAVAWSNKSDFACANAFNNSIIPEDTFFPSPESSCDVKLVEKSFETDTNLNFQNLSVIGFRILLLKVAGFNLLMTLRLWSS

SEQ ID NO: 76 - protein, 309 aa, synthetic construct
MLLLLLLLGPGSGLGAVVSQHPSWVICKSGTSVKIECRSLDFQATTMFWYRQFPKQSLMLMATSNEGSKATYEQGVEKDKFLINHASLTLSTLTVTSAHPEDSSFYICSARDIKAQQWNIQYFGAGTRLSVLEDLKNVFPPEVAVFEPSEAEISHTQKATLVCLATGFYPDHVELSWWVNGKEVHSGVSTDPQPLKEQPALNDSRYCLSSRLRVSATFWQNPRNHFRCQVQFYGLSENDEWTQDRAKPVTQIVSAEAWGRADCGFTSESYQQGVLSATILYEILLGKATLYAVLVSALVLMAMVKRKDF

SEQ ID NO: 77 - protein, 609 aa, synthetic construct
MEKNPLAAPLLILWFHLDCVSSILNVEQSPQSLHVQEGDSTNFTCSFPSSNFYALHWYRWETAKSPEALFVMTLNGDEKKKGRISATLNTKEGYSYLYIKGSQPEDSATYLCARNYGQNFVFGPGTRLSVLPYIQNPDPAVYQLRDSKSSDKSVCLFTDFDSQTNVSQSKDSDVYITDKTVLDMRSMDFKSNSAVAWSNKSDFACANAFNNSIIPEDTFFPSPESSCDVKLVEKSFETDTNLNFQNLSVIGFRILLLKVAGFNLLMTLRLWSSRAKRSGSGATNFSLLKQAGDVEENPGPMLLLLLLLGPGSGLGAVVSQHPSWVICKSGTSVKIECRSLDFQATTMFWYRQFPKQSLMLMATSNEGSKATYEQGVEKDKFLINHASLTLSTLTVTSAHPEDSSFYICSARDIKAQQWNIQYFGAGTRLSVLEDLKNVFPPEVAVFEPSEAEISHTQKATLVCLATGFYPDHVELSWWVNGKEVHSGVSTDPQPLKEQPALNDSRYCLSSRLRVSATFWQNPRNHFRCQVQFYGLSENDEWTQDRAKPVTQIVSAEAWGRADCGFTSESYQQGVLSATILYEILLGKATLYAVLVSALVLMAMVKRKDF

SEQ ID NO: 78 - protein, 6 aa, synthetic construct
VSGLRG

SEQ ID NO: 79 - protein, 7 aa, synthetic construct
LYSAGEE

SEQ ID NO: 80 - protein, 13 aa, synthetic construct
CVITTSGTYKYIF

SEQ ID NO: 81 - protein, 5 aa, synthetic construct
MNHNS

SEQ ID NO: 82 - protein, 6 aa, synthetic construct
SASEGT

SEQ ID NO: 83 - protein, 12 aa, synthetic construct
CASTINTYEQYF

SEQ ID NO: 84 - protein, 110 aa, synthetic construct
EDQVTQSPEALRLQEGESSSLNCSYTVSGLRGLFWYRQDPGKGPEFLFTLYSAGEEKEKERLKATLTKKESFLHITAPKPEDSATYLCVITTSGTYKYIFGTGTRLKVLA

SEQ ID NO: 85 - protein, 109 aa, synthetic construct
GVTQTPKFQVLKTGQSMTLQCAQDMNHNSMYWYRQDPGMGLRLIYYSASEGTTDKGEVPNGYNVSRLNKREFSLRLESAAPSQTSVYFCASTINTYEQYFGPGTRLTVT

SEQ ID NO: 86 - protein, 272 aa, synthetic construct
MEKMLECAFIVLWLQLGWLSGEDQVTQSPEALRLQEGESSSLNCSYTVSGLRGLFWYRQDPGKGPEFLFTLYSAGEEKEKERLKATLTKKESFLHITAPKPEDSATYLCVITTSGTYKYIFGTGTRLKVLANIQNPDPAVYQLRDSKSSDKSVCLFTDFDSQTNVSQSKDSDVYITDKTVLDMRSMDFKSNSAVAWSNKSDFACANAFNNSIIPEDTFFPSPESSCDVKLVEKSFETDTNLNFQNLSVIGFRILLLKVAGFNLLMTLRLWSS

SEQ ID NO: 87 - protein, 307 aa, synthetic construct
MSIGLLCCVAFSLLWASPVNAGVTQTPKFQVLKTGQSMTLQCAQDMNHNSMYWYRQDPGMGLRLIYYSASEGTTDKGEVPNGYNVSRLNKREFSLRLESAAPSQTSVYFCASTINTYEQYFGPGTRLTVTEDLKNVFPPEVAVFEPSEAEISHTQKATLVCLATGFYPDHVELSWWVNGKEVHSGVSTDPQPLKEQPALNDSRYCLSSRLRVSATFWQNPRNHFRCQVQFYGLSENDEWTQDRAKPVTQIVSAEAWGRADCGFTSESYQQGVLSATILYEILLGKATLYAVLVSALVLMAMVKRKDF

SEQ ID NO: 88 - protein, 606 aa, synthetic construct
MEKMLECAFIVLWLQLGWLSGEDQVTQSPEALRLQEGESSSLNCSYTVSGLRGLFWYRQDPGKGPEFLFTLYSAGEEKEKERLKATLTKKESFLHITAPKPEDSATYLCVITTSGTYKYIFGTGTRLKVLANIQNPDPAVYQLRDSKSSDKSVCLFTDFDSQTNVSQSKDSDVYITDKTVLDMRSMDFKSNSAVAWSNKSDFACANAFNNSIIPEDTFFPSPESSCDVKLVEKSFETDTNLNFQNLSVIGFRILLLKVAGFNLLMTLRLWSSRAKRSGSGATNFSLLKQAGDVEENPGPMSIGLLCCVAFSLLWASPVNAGVTQTPKFQVLKTGQSMTLQCAQDMNHNSMYWYRQDPGMGLRLIYYSASEGTTDKGEVPNGYNVSRLNKREFSLRLESAAPSQTSVYFCASTINTYEQYFGPGTRLTVTEDLKNVFPPEVAVFEPSEAEISHTQKATLVCLATGFYPDHVELSWWVNGKEVHSGVSTDPQPLKEQPALNDSRYCLSSRLRVSATFWQNPRNHFRCQVQFYGLSENDEWTQDRAKPVTQIVSAEAWGRADCGFTSESYQQGVLSATILYEILLGKATLYAVLVSALVLMAMVKRKDF

SEQ ID NO: 89 - protein, 9 aa, synthetic construct
ATVQGQNLK

SEQ ID NO: 90 - protein, 7 aa, synthetic construct
TSESDYY

SEQ ID NO: 91 - protein, 8 aa, synthetic construct
QEAYKQQN

SEQ ID NO: 92 - protein, 16 aa, synthetic construct
CAYRSFYTGANSKLTF

SEQ ID NO: 93 - protein, 5 aa, synthetic construct
SGHDT

SEQ ID NO: 94 - protein, 6 aa, synthetic construct
YYEEEE

SEQ ID NO: 95 - protein, 16 aa, synthetic construct
CASSLYGGPGDQPQHF

SEQ ID NO: 96 - protein, 116 aa, synthetic construct
QTVTQSQPEMSVQEAETVTLSCTYDTSESDYYLFWYKQPPSRQMILVIRQEAYKQQNATENRFSVNFQKAAKSFSLKISDSQLGDAAMYFCAYRSFYTGANSKLTFGKGITLSVRP

SEQ ID NO: 97 - protein, 113 aa, synthetic construct
GVTQSPTHLIKTRGQQVTLRCSPKSGHDTVSWYQQALGQGPQFIFQYYEEEERQRGNFPDRFSGHQFPNYSSELNVNALLLGDSALYLCASSLYGGPGDQPQHFGDGTRLSIL

SEQ ID NO: 98 - protein, 278 aa, synthetic construct
MACPGFLWALVISTCLEFSMAQTVTQSQPEMSVQEAETVTLSCTYDTSESDYYLFWYKQPPSRQMILVIRQEAYKQQNATENRFSVNFQKAAKSFSLKISDSQLGDAAMYFCAYRSFYTGANSKLTFGKGITLSVRPDIQNPDPAVYQLRDSKSSDKSVCLFTDFDSQTNVSQSKDSDVYITDKTVLDMRSMDFKSNSAVAWSNKSDFACANAFNNSIIPEDTFFPSPESSCDVKLVEKSFETDTNLNFQNLSVIGFRILLLKVAGFNLLMTLRLWSS

SEQ ID NO: 99 - protein, 311 aa, synthetic construct
MGPGLLCWALLCLLGAGLVDAGVTQSPTHLIKTRGQQVTLRCSPKSGHDTVSWYQQALGQGPQFIFQYYEEEERQRGNFPDRFSGHQFPNYSSELNVNALLLGDSALYLCASSLYGGPGDQPQHFGDGTRLSILEDLNKVFPPEVAVFEPSEAEISHTQKATLVCLATGFFPDHVELSWWVNGKEVHSGVSTDPQPLKEQPALNDSRYCLSSRLRVSATFWQNPRNHFRCQVQFYGLSENDEWTQDRAKPVTQIVSAEAWGRADCGFTSVSYQQGVLSATILYEILLGKATLYAVLVSALVLMAMVKRKDF

SEQ ID NO: 100 - protein, 616 aa, synthetic construct
MACPGFLWALVISTCLEFSMAQTVTQSQPEMSVQEAETVTLSCTYDTSESDYYLFWYKQPPSRQMILVIRQEAYKQQNATENRFSVNFQKAAKSFSLKISDSQLGDAAMYFCAYRSFYTGANSKLTFGKGITLSVRPDIQNPDPAVYQLRDSKSSDKSVCLFTDFDSQTNVSQSKDSDVYITDKTVLDMRSMDFKSNSAVAWSNKSDFACANAFNNSIIPEDTFFPSPESSCDVKLVEKSFETDTNLNFQNLSVIGFRILLLKVAGFNLLMTLRLWSSRAKRSGSGATNFSLLKQAGDVEENPGPMGPGLLCWALLCLLGAGLVDAGVTQSPTHLIKTRGQQVTLRCSPKSGHDTVSWYQQALGQGPQFIFQYYEEEERQRGNFPDRFSGHQFPNYSSELNVNALLLGDSALYLCASSLYGGPGDQPQHFGDGTRLSILEDLNKVFPPEVAVFEPSEAEISHTQKATLVCLATGFFPDHVELSWWVNGKEVHSGVSTDPQPLKEQPALNDSRYCLSSRLRVSATFWQNPRNHFRCQVQFYGLSENDEWTQDRAKPVTQIVSAEAWGRADCGFTSVSYQQGVLSATILYEILLGKATLYAVLVSALVLMAMVKRKDF

SEQ ID NO: 101 - protein, 6 aa, synthetic construct
NSASQS

SEQ ID NO: 102 - protein, 6 aa, synthetic construct
VYSSGN

SEQ ID NO: 103 - protein, 13 aa, synthetic construct
CVVHSGGSYIPTF

SEQ ID NO: 104 - protein, 5 aa, synthetic construct
MNHNY

SEQ ID NO: 105 - protein, 6 aa, synthetic construct
SVGAGI

SEQ ID NO: 106 - protein, 15 aa, synthetic construct
CASAQTIGAYNEQFF

SEQ ID NO: 107 - protein, 111 aa, synthetic construct
QRKEVEQDPGPFNVPEGATVAFNCTYSNSASQSFFWYRQDCRKEPKLLMSVYSSGNEDGRFTAQLNRASQYISLLIRDSKLSDSATYLCVVHSGGSYIPTFGRGTSLIVHP

SEQ ID NO: 108 - protein, 112 aa, synthetic construct
GVTQTPKFRILKIGQSMTLQCTQDMNHNYMYWYRQDPGMGLKLIYYSVGAGITDKGEVPNGYNVSRSTTEDFPLRLELAAPSQTSVYFCASAQTIGAYNEQFFGPGTRLTVL

SEQ ID NO: 109 - protein, 272 aa, synthetic construct
MISLRVLLVILWLQLSWVWSQRKEVEQDPGPFNVPEGATVAFNCTYSNSASQSFFWYRQDCRKEPKLLMSVYSSGNEDGRFTAQLNRASQYISLLIRDSKLSDSATYLCVVHSGGSYIPTFGRGTSLIVHPYIQNPDPAVYQLRDSKSSDKSVCLFTDFDSQTNVSQSKDSDVYITDKTVLDMRSMDFKSNSAVAWSNKSDFACANAFNNSIIPEDTFFPSPESSCDVKLVEKSFETDTNLNFQNLSVIGFRILLLKVAGFNLLMTLRLWSS

SEQ ID NO: 110 - protein, 310 aa, synthetic construct
MSISLLCCAAFPLLWAGPVNAGVTQTPKFRILKIGQSMTLQCTQDMNHNYMYWYRQDPGMGLKLIYYSVGAGITDKGEVPNGYNVSRSTTEDFPLRLELAAPSQTSVYFCASAQTIGAYNEQFFGPGTRLTVLEDLKNVFPPEVAVFEPSEAEISHTQKATLVCLATGFYPDHVELSWWVNGKEVHSGVSTDPQPLKEQPALNDSRYCLSSRLRVSATFWQNPRNHFRCQVQFYGLSENDEWTQDRAKPVTQIVSAEAWGRADCGFTSESYQQGVLSATILYEILLGKATLYAVLVSALVLMAMVKRKDF

SEQ ID NO: 111 - protein, 609 aa, synthetic construct
MISLRVLLVILWLQLSWVWSQRKEVEQDPGPFNVPEGATVAFNCTYSNSASQSFFWYRQDCRKEPKLLMSVYSSGNEDGRFTAQLNRASQYISLLIRDSKLSDSATYLCVVHSGGSYIPTFGRGTSLIVHPYIQNPDPAVYQLRDSKSSDKSVCLFTDFDSQTNVSQSKDSDVYITDKTVLDMRSMDFKSNSAVAWSNKSDFACANAFNNSIIPEDTFFPSPESSCDVKLVEKSFETDTNLNFQNLSVIGFRILLLKVAGFNLLMTLRLWSSRAKRSGSGATNFSLLKQAGDVEENPGPMSISLLCCAAFPLLWAGPVNAGVTQTPKFRILKIGQSMTLQCTQDMNHNYMYWYRQDPGMGLKLIYYSVGAGITDKGEVPNGYNVSRSTTEDFPLRLELAAPSQTSVYFCASAQTIGAYNEQFFGPGTRLTVLEDLKNVFPPEVAVFEPSEAEISHTQKATLVCLATGFYPDHVELSWWVNGKEVHSGVSTDPQPLKEQPALNDSRYCLSSRLRVSATFWQNPRNHFRCQVQFYGLSENDEWTQDRAKPVTQIVSAEAWGRADCGFTSESYQQGVLSATILYEILLGKATLYAVLVSALVLMAMVKRKDF